European Patent Application EP 4 159 768 A1, published April 5, 2023. Title: Enhanced synthetic T cell receptor and antigen receptor. Applicant: China Immunotech (Beijing) Biotechnology Co., Ltd. Tsinghua University. The sequence listing filed with the application follows.

SEQUENCE LISTING (60 sequences)

SEQ ID NO: 1 - protein, 141 aa, Homo sapiens
DIQNPDPAVYQLRDSKSSDKSVCLFTDFDSQTNVSQSKDSDVYITDKTVLDMRSMDFKSNSAVAWSNKSDFACANAFNNSIIPEDTFFPSPESSCDVKLVEKSFETDTNLNFQNLSVIGFRILLLKVAGFNLLMTLRLWSS

SEQ ID NO: 2 - protein, 176 aa, Homo sapiens
DLKNVFPPEVAVFEPSEAEISHTQKATLVCLATGFYPDHVELSWWVNGKEVHSGVSTDPQPLKEQPALNDSRYCLSSRLRVSATFWQNPRNHFRCQVQFYGLSENDEWTQDRAKPVTQIVSAEAWGRADCGFTSESYQQGVLSATILYEILLGKATLYAVLVSALVLMAMVKRKDF

SEQ ID NO: 3 - protein, 137 aa, Mus musculus
DIQNPEPAVYQLKDPRSQDSTLCLFTDFDSQINVPKTMESGTFITDKTVLDMKAMDSKSNGAIAWSNQTSFTCQDIFKETNATYPSSDVPCDATLTEKSFETDMNLNFQNLSVMGLRILLLKVAGFNLLMTLRLWSS

SEQ ID NO: 4 - protein, 172 aa, Mus musculus
DLRNVTPPKVSLFEPSKAEIANKQKATLVCLARGFFPDHVELSWWVNGKEVHSGVSTDPQAYKESNYSYCLSSRLRVSATFWHNPRNHFRCQVQFHGLSEEDKWPEGSPKPVTQNISAEAWGRADCGITSASYQQGVLSATILYEILLGKATLYAVLVSTLVVMAMVKRKNS

SEQ ID NO: 5 - protein, 137 aa, Artificial Sequence
  Artificial Sequence
DIQNPEPAVYQLKDPRSQDSTLCLFTDFDSQINVPKTMESGTFITDKCVLDMKAMDSKSNGAIAWSNQTSFTCQDIFKETNATYPSSDVPCDATLTEKSFETDMNLNFQNLSVMGLRILLLKVAGFNLLMTLRLWSS

SEQ ID NO: 6 - protein, 172 aa, Artificial Sequence
  Artificial Sequence
DLRNVTPPKVSLFEPSKAEIANKQKATLVCLARGFFPDHVELSWWVNGKEVHSGVCTDPQAYKESNYSYCLSSRLRVSATFWHNPRNHFRCQVQFHGLSEEDKWPEGSPKPVTQNISAEAWGRADCGITSASYQQGVLSATILYEILLGKATLYAVLVSTLVVMAMVKRKNS

SEQ ID NO: 7 - protein, 137 aa, Artificial Sequence
  Artificial Sequence
DIQNPEPAVYQLKDPRSQDSTLCLFTDFDSQINVPKTMESGTFITDKTVLDMKAMDSKSNGAIAWSNQTSFTCQDIFKETNATYPSSDVPCDATLTEKSFETDMNLNFQNLLVIVLRILLLKVAGFNLLMTLRLWSS

SEQ ID NO: 8 - protein, 137 aa, Artificial Sequence
  Artificial Sequence
DIQNPEPAVYQLKDPRSQDSTLCLFTDFDSQINVPKTMESGTFITDKCVLDMKAMDSKSNGAIAWSNQTSFTCQDIFKETNATYPSSDVPCDATLTEKSFETDMNLNFQNLLVIVLRILLLRVAGFNLLMTLRLWSS

SEQ ID NO: 9 - protein, 172 aa, Artificial Sequence
  Artificial Sequence
DLRNVTPPKVSLFEPSKAEIANKQKATLVCLARGFFPDHVELSWWVNGKEVHSGVCTDPQAYKESNYSYCLSSRLRVSATFWHNPRNHFRCQVQFHGLSEEDKWPEGSPKPVTQNISAEAWGRADCGITSASYQQGVLSATILYEILLGRATLYAVLVSTLVVMAMVRRRNS

SEQ ID NO: 10 - protein, 61 aa, Artificial Sequence
  Artificial Sequence
KKVAKKPTNKAPHPKQEPQEINFPDDLPGSNTAAPVQETLHGCQPVTQEDGKESRISVQER

SEQ ID NO: 11 - protein, 37 aa, Artificial Sequence
  Artificial Sequence
RRDQRLPPDAHKPPGGGSFRTPIQEEQADAHSTLAKI

SEQ ID NO: 12 - protein, 34 aa, Artificial Sequence
  Artificial Sequence
KKKYSSSVHDPNGEYMFMRAVNTAKKSRLTDVTL

SEQ ID NO: 13 - protein, 41 aa, Artificial Sequence
  Artificial Sequence
RSKRSRLLHSDYMNMTPRRPGPTRKHYQPYAPPRDFAAYRS

SEQ ID NO: 14 - protein, 42 aa, Artificial Sequence
  Artificial Sequence
KRGRKKLLYIFKQPFMRPVQTTQEEDGCSCRFPEEEEGGCEL

SEQ ID NO: 15 - protein, 48 aa, Artificial Sequence
  Artificial Sequence
QRRKYRSNKGESPVEPAEPCRYSCPREEEGSTIPIQEDYRKPEPACSP

SEQ ID NO: 16 - protein, 5 aa, Artificial Sequence
  Artificial Sequence
GGGGS

SEQ ID NO: 17 - protein, 10 aa, Artificial Sequence
  Artificial Sequence
GGGGSGGGGS

SEQ ID NO: 18 - protein, 15 aa, Artificial Sequence
  Artificial Sequence
GGGGSGGGGSGGGGS

SEQ ID NO: 19 - protein, 20 aa, Artificial Sequence
  Artificial Sequence
GGGGSGGGGSGGGGSGGGGS

SEQ ID NO: 20 - protein, 25 aa, Artificial Sequence
  Artificial Sequence
GGGGSGGGGSGGGGSGGGGSGGGGS

SEQ ID NO: 21 - protein, 30 aa, Artificial Sequence
  Artificial Sequence
GGGGSGGGGSGGGGSGGGGSGGGGSGGGGS

SEQ ID NO: 22 - protein, 35 aa, Artificial Sequence
  Artificial Sequence
GGGGSGGGGSGGGGSGGGGSGGGGSGGGGSGGGGS

SEQ ID NO: 23 - protein, 40 aa, Artificial Sequence
  Artificial Sequence
GGGGSGGGGSGGGGSGGGGSGGGGSGGGGSGGGGSGGGGS

SEQ ID NO: 24 - protein, 45 aa, Artificial Sequence
  Artificial Sequence
GGGGSGGGGSGGGGSGGGGSGGGGSGGGGSGGGGSGGGGSGGGGS

SEQ ID NO: 25 - protein, 50 aa, Artificial Sequence
  Artificial Sequence
GGGGSGGGGSGGGGSGGGGSGGGGSGGGGSGGGGSGGGGSGGGGSGGGGS

SEQ ID NO: 26 - protein, 135 aa, Artificial Sequence
  Artificial Sequence
DIQNPEPAVYQLKDPRSQDSTLCLFTDFDSQINVPKTMESGTFITDKCVLDMKAMDSKSNGAIAWSNQTSFTCQDIFKETNATYPSSDVPCDATLTEKSFETDMNLNFQNLLVIVLRILLLKVAGFNLLMTLRLW

SEQ ID NO: 27 - protein, 166 aa, Artificial Sequence
  Artificial Sequence
DLRNVTPPKVSLFEPSKAEIANKQKATLVCLARGFFPDHVELSWWVNGKEVHSGVCTDPQAYKESNYSYCLSSRLRVSATFWHNPRNHFRCQVQFHGLSEEDKWPEGSPKPVTQNISAEAWGRADCGITSASYQQGVLSATILYEILLGKATLYAVLVSTLVVMAM

SEQ ID NO: 28 - protein, 182 aa, Homo sapiens
MEQGKGLAVLILAIILLQGTLAQSIKGNHLVKVYDYQEDGSVLLTCDAEAKNITWFKDGKMIGFLTEDKKKWNLGSNAKDPRGMYQCKGSQNKSKPLQVYYRMCQNCIELNAATISGFLFAEIVSIFVLAVGVYFIAGQDGVRQSRASDKQTLLPNDQLYQPLKDREDDQYSHLQGNQLRRN

SEQ ID NO: 29 - protein, 171 aa, Homo sapiens
MEHSTFLSGLVLATLLSQVSPFKIPIEELEDRVFVNCNTSITWVEGTVGTLLSDITRLDLGKRILDPRGIYRCNGTDIYKDKESTVQVHYRMCQSCVELDPATVAGIIVTDVIATLLLALGVFCFAGHETGRLSGAADTQALLRNDQVYQPLRDRDDAQYSHLGGNWARNK

SEQ ID NO: 30 - protein, 207 aa, Homo sapiens
MQSGTHWRVLGLCLLSVGVWGQDGNEEMGGITQTPYKVSISGTTVILTCPQYPGSEILWQHNDKNIGGDEDDKNIGSDEDHLSLKEFSELEQSGYYVCYPRGSKPEDANFYLYLRARVCENCMEMDVMSVATIVIVDICITGGLLLLVYYWSKNRKAKAKPVTRGAGAGGRQRGQNKERPPPVPNPDYEPIRKGQRDLYSGLNQRRI

SEQ ID NO: 31 - protein, 163 aa, Homo sapiens
MKWKALFTAAILQAQLPITEAQSFGLLDPKLCYLLDGILFIYGVILTALFLRVKFSRSADAPAYQQGQNQLYNELNLGRREEYDVLDKRRGRDPEMGGKPRRKNPQEGLYNELQKDKMAEAYSEIGMKGERRRGKGHDGLYQGLSTATKDTYDALHMQALPPR

SEQ ID NO: 32 - protein, 94 aa, Homo sapiens
NCRNTGPWLKKVLKCNTPDPSKFFSQLSSEHGGDVQKWLSSPFPSSSFSPGGLAPEISPLEVLERDKVTQLLPLNTDAYLSLQELQGQDPTHLV

SEQ ID NO: 33 - protein, 195 aa, Homo sapiens
KKRIKPIVWPSLPDHKKTLEHLCKKPRKNLNVSFNPESFLDCQIHRVDDIQARDEVEGFLQDTFPQQLEESEKQRLGGDVQSPNCPSEDVVITPESFGRDSSLTCLAGNVSACDAPILSSSRSLDCRESGKNGPHVYQDLLLSLGTTNSTLPPPFSLQSGILTLNPVAQGQPILTSLGSNQEEAYVTMSSFYQNQ

SEQ ID NO: 34 - protein, 285 aa, Homo sapiens
SLKTHPLWRLWKKIWAVPSPERFFMPLYKGCSGDFKKWVGAPFTGSSLELGPWSPEVPSTLEVYSCHPPRSPAKRLQLTELQEPAELVESDGVPKPSFWPTAQNSGGSAYSEERDRPYGLVSIDTVTVLDAEGPCTWPCSCEDDGYPALDLDAGLEPSPGLEDPLLDAGTTVLSCGCVSAGSPGLGGPLGSLLDRLKPPLADGEDWAGGLPWGGRSPGGVSESEAGSPLAGLDMDTFDSGFVGSDCSSPVECDFTSPGDEGPPRSYLRQWVVIPPPLSSPGPQAS

SEQ ID NO: 35 - protein, 4 aa, Homo sapiens
YRHQ

SEQ ID NO: 36 - protein, 103 aa, Artificial Sequence
  Artificial Sequence
NCRNTGPWLKKVLKCNTPDPSKFFSQLSSEHGGDVQKWLSSPFPSSSFSPGGLAPEISPLEVLERDKVTQLLPLNTDAYLSLQELQGQDPTHLVGGGGSYRHQ

SEQ ID NO: 37 - protein, 204 aa, Artificial Sequence
  Artificial Sequence
KKRIKPIVWPSLPDHKKTLEHLCKKPRKNLNVSFNPESFLDCQIHRVDDIQARDEVEGFLQDTFPQQLEESEKQRLGGDVQSPNCPSEDVVITPESFGRDSSLTCLAGNVSACDAPILSSSRSLDCRESGKNGPHVYQDLLLSLGTTNSTLPPPFSLQSGILTLNPVAQGQPILTSLGSNQEEAYVTMSSFYQNQGGGGSYRHQ

SEQ ID NO: 38 - protein, 244 aa, Artificial Sequence
  Artificial Sequence
EIVLTQSPATLSLSPGERATLSCRASQSVSSYLAWYQQKPGQAPRLLIYDASNRATGIPARFSGSGSGTDFTLTISSLEPEDFAVYYCQQRSNWPITFGQGTRLEIKGGGGSGGGGSGGGGSEVQLVESGGGLVQPGRSLRLSCAASGFTFNDYAMHWVRQAPGKGLEWVSTISWNSGSIGYADSVKGRFTISRDNAKKSLYLQMNSLRAEDTALYYCAKDIQYGNYYYGMDVWGQGTTVTVSS

SEQ ID NO: 39 - protein, 242 aa, Artificial Sequence
  Artificial Sequence
DIQMTQTTSSLSASLGDRVTISCRASQDISKYLNWYQQKPDGTVKLLIYHTSRLHSGVPSRFSGSGSGTDYSLTISNLEQEDIATYFCQQGNTLPYTFGGGTKLEITGGGGSGGGGSGGGGSEVKLQESGPGLVAPSQSLSVTCTVSGVSLPDYGVSWIRQPPRKGLEWLGVIWGSETTYYNSALKSRLTIIKDNSKSQVFLKMNSLQTDDTAIYYCAKHYYYGGSYAMDYWGQGTSVTVSS

SEQ ID NO: 40 - protein, 225 aa, Artificial Sequence
  Artificial Sequence
MASSEDVIKEFMRFKVRMEGSVNGHEFEIEGEGEGRPYEGTQTAKLKVTKGGPLPFAWDILSPQFQYGSKAYVKHPADIPDYLKLSFPEGFKWERVMNFEDGGVVTVTQDSSLQDGEFIYKVKLRGTNFPSDGPVMQKKTMGWEASTERMYPEDGALKGEIKMRLKLKDGGHYDAEVKTTYMAKKPVQLPGAYKTDIKLDITSHNEDYTIVEQYERAEGRHSTGA

SEQ ID NO: 41 - protein, 137 aa, Artificial Sequence
  Artificial Sequence
DIQNPEPAVYQLKDPRSQDSTLCLFTDFDSQINVPKTMESGTFITDKCVLDMKAMDSKSNGAIAWSNQTSFTCQDIFKETNATYPSSDVPCDATLTEKSFETDMNLNFQNLLVIVLRILLLKVAGFNLLMTLRLWSS

SEQ ID NO: 42 - protein, 133 aa, Artificial Sequence
  Artificial Sequence
DIQNPDPAVYQLRDDSTLCLFTDFDSQINVPKTMESGTFITDKCVLDMKAMDSKSNGAIAWSNQTSFTCQDIFKETNATYPSSDVPCDATLTEKSFETDMNLNFQNLLVIVLRILLLKVAGFNLLMTLRLWSS

SEQ ID NO: 43 - protein, 166 aa, Artificial Sequence
  Artificial Sequence
DLKNVFPPEVAVFEPSAEIATLVCLARGFFPDHVELSWWVNGKEVHSGVCTDPQAYKESNYSYCLSSRLRVSATFWHNPRNHFRCQVQFHGLSEEDKWPEGSPKPVTQNISAEAWGRADCGITSASYQQGVLSATILYEILLGKATLYAVLVSTLVVMAMVKRKNS

SEQ ID NO: 44 - protein, 120 aa, Artificial Sequence
  Artificial Sequence
EVKLQESGPGLVAPSQSLSVTCTVSGVSLPDYGVSWIRQPPRKGLEWLGVIWGSETTYYNSALKSRLTIIKDNSKSQVFLKMNSLQTDDTAIYYCAKHYYYGGSYAMDYWGQGTSVTVSS

SEQ ID NO: 45 - protein, 107 aa, Artificial Sequence
  Artificial Sequence
DIQMTQTTSSLSASLGDRVTISCRASQDISKYLNWYQQKPDGTVKLLIYHTSRLHSGVPSRFSGSGSGTDYSLTISNLEQEDIATYFCQQGNTLPYTFGGGTKLEIT

SEQ ID NO: 46 - protein, 113 aa, Artificial Sequence
  Artificial Sequence
QVQLQQSGAELVRPGASVKLSCKALGFIFTDYEIHWVKQTPVHGLEWIGAFHPGSGGSAYNQKFKGKATLTADKSSSTAYMELSSLTFEDSAVYHCTRQLGPDWGQGTLVTVS

SEQ ID NO: 47 - protein, 112 aa, Artificial Sequence
  Artificial Sequence
DVVMTQTPLTLSVTIGQPASISCKSSQSLLESDGKTYLNWLLQRPGQSPKRLIYLVSKLDSGVPDRFTGSGSGTDFTLRISRVEAEDLGVYYCWQGTQFPWTFGGGTKLEIK

SEQ ID NO: 48 - protein, 131 aa, Artificial Sequence
  Artificial Sequence
DIQNPDPAVYQLRDDSTLCLFTDFDSQINVPKTMESGTFITDKCVLDMKAMDSKSNGAIAWSNQTSFTCQDIFKETNATYPSSDVPCDATLTEKSFETDMNLNFQNLLVIVLRILLLKVAGFNLLMTLRLW

SEQ ID NO: 49 - protein, 160 aa, Artificial Sequence
  Artificial Sequence
DLKNVFPPEVAVFEPSAEIATLVCLARGFFPDHVELSWWVNGKEVHSGVCTDPQAYKESNYSYCLSSRLRVSATFWHNPRNHFRCQVQFHGLSEEDKWPEGSPKPVTQNISAEAWGRADCGITSASYQQGVLSATILYEILLGKATLYAVLVSTLVVMAM

SEQ ID NO: 50 - protein, 173 aa, Homo sapiens
DKQLDADVSPKPTIFLPSIAETKLQKAGTYLCLLEKFFPDVIKIHWQEKKSNTILGSQEGNTMKTNDTYMKFSWLTVPEKSLDKEHRCIVRHENNKNGVDQEIIFPPIKTDVITMDPKDNCSKDANDTLLLQLTNTSAYYMYLLLLLKSVVYFAIITCCLLRRTAFCCNGEKS

SEQ ID NO: 51 - protein, 172 aa, Mus musculus
  misc_feature (1)..(1): Xaa can be any naturally occurring amino acid
XKRLDADISPKPTIFLPSVAETNLHKTGTYLCLLEKFFPDVIRVYWKEKDGNTILDSQEGDTLKTNDTYMKFSWLTVPERAMGKEHRCIVKHENNKGGADQEIFFPSIKKVAVSTKPTTCWQDKNDVLQLQFTITSAYYTYLLLLLKSVIYLAIISFSLLRRTSVCGNEKKS

SEQ ID NO: 52 - protein, 154 aa, Homo sapiens
  misc_feature (1)..(1): Xaa can be any naturally occurring amino acid
XSQPHTKPSVFVMKNGTNVACLVKEFYPKDIRINLVSSKKITEFDPAIVISPSGKYNAVKLGKYEDSNSVTCSVQHDNKTVHSTDFEVKTDSTDHVKPKETENTKQPSKSCHKPKAIVHTEKVNMMSLTVLGLRMLFAKTVAVNFLLTAKLFFL

SEQ ID NO: 53 - protein, 153 aa, Mus musculus
  misc_feature (1)..(1): Xaa can be any naturally occurring amino acid
XSQPPAKPSVFIMKNGTNVACLVKDFYPKEVTISLRSSKKIVEFDPAIVISPSGKYSAVKLGQYGDSNSVTCSVQHNSETVHSTDFEPYANSFNNEKLPEPENDTQISEPCYGPRVTVHTEKVNMMSLTVLGLRLLFAKTIAINFLLTVKLFF

SEQ ID NO: 54 - protein, 123 aa, Artificial Sequence
  Artificial Sequence
AVQLVESGGGLVQPGRSLRLSCAASGFTFGDYTMHWVRQAPGKGLEWVSGISWNSGSIGYADSVKGRFTISRDNAKNSLYLQMNSLRAEDTALYYCTKDNQYGSGSTYGLGVWGQGTLVTVSS

SEQ ID NO: 55 - protein, 107 aa, Artificial Sequence
  Artificial Sequence
EIVLTQSPATLSLSPGERATLSCRASQSVSSYLAWYQQKPGQAPRLLIYDASNRATGIPARFSGSGSGTDFTLTISSLEPEDFAVYYCQQRSNWPLTFGGGTKVEIK

SEQ ID NO: 56 - protein, 122 aa, Artificial Sequence
  Artificial Sequence
EVQLVESGGGLVQPGRSLRLSCAASGFTFNDYAMHWVRQAPGKGLEWVSTISWNSGSIGYADSVKGRFTISRDNAKKSLYLQMNSLRAEDTALYYCAKDIQYGNYYYGMDVWGQGTTVTVSS

SEQ ID NO: 57 - protein, 107 aa, Artificial Sequence
  Artificial Sequence
EIVLTQSPATLSLSPGERATLSCRASQSVSSYLAWYQQKPGQAPRLLIYDASNRATGIPARFSGSGSGTDFTLTISSLEPEDFAVYYCQQRSNWPITFGQGTRLEIK

SEQ ID NO: 58 - protein, 918 aa, Artificial Sequence
  Artificial Sequence
MLLLVTSLLLCELPHPAFLLIPEIVLTQSPATLSLSPGERATLSCRASQSVSSYLAWYQQKPGQAPRLLIYDASNRATGIPARFSGSGSGTDFTLTISSLEPEDFAVYYCQQRSNWPLTFGGGTKVEIKGGGGSGGGGSGGGGSAVQLVESGGGLVQPGRSLRLSCAASGFTFGDYTMHWVRQAPGKGLEWVSGISWNSGSIGYADSVKGRFTISRDNAKNSLYLQMNSLRAEDTALYYCTKDNQYGSGSTYGLGVWGQGTLVTVSSEDLRNVTPPKVSLFEPSKAEIANKQKATLVCLARGFFPDHVELSWWVNGKEVHSGVCTDPQAYKESNYSYCLSSRLRVSATFWHNPRNHFRCQVQFHGLSEEDKWPEGSPKPVTQNISAEAWGRADCGITSASYQQGVLSATILYEILLGKATLYAVLVSTLVVMAMVKRKNSRRKRSGSGATNFSLLKQAGDVEENPGPMLLLVTSLLLCELPHPAFLLIPDIQMTQTTSSLSASLGDRVTISCRASQDISKYLNWYQQKPDGTVKLLIYHTSRLHSGVPSRFSGSGSGTDYSLTISNLEQEDIATYFCQQGNTLPYTFGGGTKLEITGGGGSGGGGSGGGGSEVKLQESGPGLVAPSQSLSVTCTVSGVSLPDYGVSWIRQPPRKGLEWLGVIWGSETTYYNSALKSRLTIIKDNSKSQVFLKMNSLQTDDTAIYYCAKHYYYGGSYAMDYWGQGTSVTVSSDIQNPEPAVYQLKDPRSQDSTLCLFTDFDSQINVPKTMESGTFITDKCVLDMKAMDSKSNGAIAWSNQTSFTCQDIFKETNATYPSSDVPCDATLTEKSFETDMNLNFQNLLVIVLRILLLKVAGFNLLMTLRLWGGGGSGGGGSGGGGSRRDQRLPPDAHKPPGGGSFRTPIQEEQADAHSTLAKI

SEQ ID NO: 59 - protein, 429 aa, Artificial Sequence
  Artificial Sequence
DIQMTQTTSSLSASLGDRVTISCRASQDISKYLNWYQQKPDGTVKLLIYHTSRLHSGVPSRFSGSGSGTDYSLTISNLEQEDIATYFCQQGNTLPYTFGGGTKLEITGGGGSGGGGSGGGGSEVKLQESGPGLVAPSQSLSVTCTVSGVSLPDYGVSWIRQPPRKGLEWLGVIWGSETTYYNSALKSRLTIIKDNSKSQVFLKMNSLQTDDTAIYYCAKHYYYGGSYAMDYWGQGTSVTVSSDIQNPEPAVYQLKDPRSQDSTLCLFTDFDSQINVPKTMESGTFITDKCVLDMKAMDSKSNGAIAWSNQTSFTCQDIFKETNATYPSSDVPCDATLTEKSFETDMNLNFQNLLVIVLRILLLKVAGFNLLMTLRLWGGGGSGGGGSGGGGSRRDQRLPPDAHKPPGGGSFRTPIQEEQADAHSTLAKI

SEQ ID NO: 60 - protein, 418 aa, Artificial Sequence
  Artificial Sequence
EIVLTQSPATLSLSPGERATLSCRASQSVSSYLAWYQQKPGQAPRLLIYDASNRATGIPARFSGSGSGTDFTLTISSLEPEDFAVYYCQQRSNWPLTFGGGTKVEIKGGGGSGGGGSGGGGSAVQLVESGGGLVQPGRSLRLSCAASGFTFGDYTMHWVRQAPGKGLEWVSGISWNSGSIGYADSVKGRFTISRDNAKNSLYLQMNSLRAEDTALYYCTKDNQYGSGSTYGLGVWGQGTLVTVSSEDLRNVTPPKVSLFEPSKAEIANKQKATLVCLARGFFPDHVELSWWVNGKEVHSGVCTDPQAYKESNYSYCLSSRLRVSATFWHNPRNHFRCQVQFHGLSEEDKWPEGSPKPVTQNISAEAWGRADCGITSASYQQGVLSATILYEILLGKATLYAVLVSTLVVMAMVKRKNS